European Patent Specification EP 4 019 027 B1, published January 22, 2025. Title: Composition for Protecting or Treating Non-alcoholic steatohepatitis comprising Exosomes derived from Precursor cell of iPSC-derived mesenchymal stem cell. Applicant: BREXOGEN INC. The sequence listing filed with the application follows.

SEQUENCE LISTING (14 sequences)

SEQ ID NO: 1 - DNA, 20 bp, Artificial Sequence
  FABP4-F
gcatggccaaacctaacatg

SEQ ID NO: 2 - DNA, 20 bp, Artificial Sequence
  FABP4-R
cctggcccagtatgaaggaa

SEQ ID NO: 3 - DNA, 24 bp, Artificial Sequence
  TNFa-F
gagctgaacaataggctgttccca

SEQ ID NO: 4 - DNA, 24 bp, Artificial Sequence
  TNFa-R
agaggctcagcaatgagtgacagt

SEQ ID NO: 5 - DNA, 20 bp, Artificial Sequence
  MCP1-F
tctgtgcctgctgctcatag

SEQ ID NO: 6 - DNA, 20 bp, Artificial Sequence
  MCP1-R
gggcattgattgcatctggc

SEQ ID NO: 7 - DNA, 24 bp, Artificial Sequence
  CHOP-F
agggagaaccaggaaacggaaaca

SEQ ID NO: 8 - DNA, 24 bp, Artificial Sequence
  CHOP-R
tcctgcttgagccgttcattctct

SEQ ID NO: 9 - DNA, 20 bp, Artificial Sequence
  ACC1-F
gctccttgtcacctgcttct

SEQ ID NO: 10 - DNA, 20 bp, Artificial Sequence
  ACC1-R
caaggccaagccatcctgta

SEQ ID NO: 11 - DNA, 20 bp, Artificial Sequence
  SREBP1-F
ggaggggtaggggccaacgc

SEQ ID NO: 12 - DNA, 20 bp, Artificial Sequence
  SREBP1-R
catgtcttcgaaagtgcaat

SEQ ID NO: 13 - DNA, 20 bp, Artificial Sequence
  IL10-F
tgaaaacaagagcaaggccg

SEQ ID NO: 14 - DNA, 20 bp, Artificial Sequence
  IL10-R
gccaccctgatgtctcagtt